European Patent Application EP 4 372 006 A1, published May 22, 2024. Title: Anti Tim-3 antibody or antibody derivative and the use thereof. Applicant: ブライトパス・バイオ株式会社. Application JP. The sequence listing filed with the application follows.

SEQUENCE LISTING (88 sequences)

SEQ ID NO: 1 - protein, 5 aa, Mus musculus
SYYMS

SEQ ID NO: 2 - protein, 17 aa, Mus musculus
TISNSGGSIYYLDSVKD

SEQ ID NO: 3 - protein, 12 aa, Mus musculus
DPYYSNYVPMDY

SEQ ID NO: 4 - protein, 11 aa, Mus musculus
KASQYVDTYVA

SEQ ID NO: 5 - protein, 7 aa, Mus musculus
SASTRHT

SEQ ID NO: 6 - protein, 9 aa, Mus musculus
AQYSSSPLT

SEQ ID NO: 7 - protein, 121 aa, Mus musculus
EVMLMESGGGLVKLGGSLKLSCAASGFTFSSYYMSWVRQTPEKRLEWVATISNSGGSIYYLDSVKDRFTISRDNAKNTLYLQMSSLNSEDTAVYYCARDPYYSNYVPMDYWGQGTSVTVSS

SEQ ID NO: 8 - protein, 107 aa, Mus musculus
SIVMTQTPKFMSTSVGDRVSVTCKASQYVDTYVAWYQQKPGQSPKPLIYSASTRHTGVPARFTGSGSGTDFTLTISNVQSEDLAEYFCAQYSSSPLTFGAGTKLELK

SEQ ID NO: 9 - protein, 5 aa, Mus musculus
DYYMD

SEQ ID NO: 10 - protein, 17 aa, Mus musculus
YIYPNNGGTSYNQKFKG

SEQ ID NO: 11 - protein, 11 aa, Mus musculus
SGYGNYYTMDY

SEQ ID NO: 12 - protein, 11 aa, Mus musculus
KASQSVGNNVA

SEQ ID NO: 13 - protein, 7 aa, Mus musculus
YASNRYT

SEQ ID NO: 14 - protein, 9 aa, Mus musculus
QQHYSSPST

SEQ ID NO: 15 - protein, 120 aa, Mus musculus
QVQLQQSGPERVKPGDSVKMSCKASGYTFTDYYMDWVKQSHGKSLEWIGYIYPNNGGTSYNQKFKGKATLTVDKSSSTAYMELHSLTSEDSAVYYCARSGYGNYYTMDYWGQGTSVTVSA

SEQ ID NO: 16 - protein, 107 aa, Mus musculus
SIVMTQTPKFMPVSAGDRVTMTCKASQSVGNNVAWYQQKPGQSPKLLIYYASNRYTGVPDRFTGSGSGTDFTFTISSVQVEDLAVYFCQQHYSSPSTFGTGTKLEIK

SEQ ID NO: 17 - protein, 5 aa, Mus musculus
DYYMD

SEQ ID NO: 18 - protein, 17 aa, Mus musculus
YIYPNNGGTSYNQKFKG

SEQ ID NO: 19 - protein, 11 aa, Mus musculus
GGYYSYYSYDY

SEQ ID NO: 20 - protein, 11 aa, Mus musculus
KASQSVGNNVA

SEQ ID NO: 21 - protein, 7 aa, Mus musculus
YASNRYT

SEQ ID NO: 22 - protein, 9 aa, Mus musculus
QQHYSSPYT

SEQ ID NO: 23 - protein, 120 aa, Mus musculus
QVQLQQSGPELVKPGDSVKMSCKASGYTFTDYYMDWVKQSHGKSLEWIGYIYPNNGGTSYNQKFKGKATLTVDKSSSTAYMELHSLTSEDSAVYYCARGGYYSYYSYDYWGQGTTLTVSS

SEQ ID NO: 24 - protein, 107 aa, Mus musculus
SIVMTQTPKFLPVSAGDRVTMTCKASQSVGNNVAWYQQKPGQSPKLLIYYASNRYTGVPDRFTGSGSGTDFTFTISSVQVEDLAVYFCQQHYSSPYTFGTGTKLEIK

SEQ ID NO: 25 - protein, 5 aa, Mus musculus
DYYMD

SEQ ID NO: 26 - protein, 17 aa, Mus musculus
YIYPNNGGTSYNQKFKG

SEQ ID NO: 27 - protein, 11 aa, Mus musculus
SGYKAYYAMDY

SEQ ID NO: 28 - protein, 11 aa, Mus musculus
KASQSVGNNVA

SEQ ID NO: 29 - protein, 7 aa, Mus musculus
YASNRYT

SEQ ID NO: 30 - protein, 9 aa, Mus musculus
QQHYSSPYT

SEQ ID NO: 31 - protein, 120 aa, Mus musculus
QIQLQQSGPELVKPGDSVKMSCKASGYTFTDYYMDWVKQSHGKSLEWIGYIYPNNGGTSYNQKFKGKATLTVDKSSSTAYMELHSLTSEDSAVYYCARSGYKAYYAMDYWGQGTTLTVSS

SEQ ID NO: 32 - protein, 107 aa, Mus musculus
SIVMTQTPKFLPVSAGDRVTMTCKASQSVGNNVAWYQQKPGQSPKLLIYYASNRYTGVPDRFTGSGSGTDFTFTISSVQVEDLAVYFCQQHYSSPYTFGSGTKLEIK

SEQ ID NO: 33 - protein, 5 aa, synthetic construct
  REGION 1..5: note = CDR1 of type d HC of 003 antibody
SYYMS

SEQ ID NO: 34 - protein, 17 aa, synthetic construct
  REGION 1..17: note = CDR2 of type d HC of 003 antibody
TISNSGGSTYYPDSVKD

SEQ ID NO: 35 - protein, 12 aa, synthetic construct
  REGION 1..12: note = CDR3 of type d HC of 003 antibody
DPYYTNYVPMDY

SEQ ID NO: 36 - protein, 121 aa, synthetic construct
  REGION 1..121: note = HC variable domain of 003_F20 antibody
EVMLMESGGGLVKLGGSLKLSCAASGFTFSSYYMSWVRQTPEKRLEWVATISNSGGSTYYPDSVKDRFTISRDNAKNTLYLQMSSLNSEDTAVYYCARDPYYTNYVPMDYWGQGTSVTVSS

SEQ ID NO: 37 - protein, 5 aa, synthetic construct
  REGION 1..5: note = CDR1 of type b HC of 003 antibody
SYYMS

SEQ ID NO: 38 - protein, 17 aa, synthetic construct
  REGION 1..17: note = CDR2 of type b HC of 003 antibody
TISNSGGSTYYPDSVKD

SEQ ID NO: 39 - protein, 12 aa, synthetic construct
  REGION 1..12: note = CDR3 of type b HC of 003 antibody
DPYYSNYVPMDY

SEQ ID NO: 40 - protein, 5 aa, synthetic construct
  REGION 1..5: note = CDR1 of type c HC of 003 antibody
SYYMS

SEQ ID NO: 41 - protein, 17 aa, synthetic construct
  REGION 1..17: note = CDR2 of type c HC of 003 antibody
TISNSGGSIYYPDSVKD

SEQ ID NO: 42 - protein, 12 aa, synthetic construct
  REGION 1..12: note = CDR3 of type c HC of 003 antibody
DPYYSNYVPMDY

SEQ ID NO: 43 - protein, 5 aa, synthetic construct
  REGION 1..5: note = CDR1 of type e HC of 003 antibody
SYYMS

SEQ ID NO: 44 - protein, 17 aa, synthetic construct
  REGION 1..17: note = CDR2 of type e HC of 003 antibody
TVSNSGGSTYYPDSVKD

SEQ ID NO: 45 - protein, 12 aa, synthetic construct
  REGION 1..12: note = CDR3 of type e HC of 003 antibody
DPYYTNYVPMDY

SEQ ID NO: 46 - protein, 11 aa, synthetic construct
  REGION 1..11: note = CDR1 of type A2 LC of 003 antibody
KASQYVGTYVA

SEQ ID NO: 47 - protein, 7 aa, synthetic construct
  REGION 1..7: note = CDR2 of type A2 LC of 003 antibody
SASTRHT

SEQ ID NO: 48 - protein, 9 aa, synthetic construct
  REGION 1..9: note = CDR3 of type A2 LC of 003 antibody
EQYSSSPLT

SEQ ID NO: 49 - protein, 121 aa, synthetic construct
  REGION 1..121: note = HC variable domain of Hu003_13 antibody
QVQLQESGGGLVKPGGSLKLSCAASGFTFSSYYMSWVRQTPDKRLEWVATISNSGGSIYYLDSVKDRFTISRDNAKNTLYLQMSSLKSEDTAMYYCARDPYYSNYVPMDYWGQGTMVTVSS

SEQ ID NO: 50 - protein, 107 aa, synthetic construct
  REGION 1..107: note = LC variable domain of Hu003_13 antibody
DIVMTQSPSFLSASVGDRVTITCKASQYVDTYVAWYQQRPGKAPKPLIYSASTRHTGVPSRFSGSGSGTEFTLTISSLQPEDFATYFCAQYSSSPLTFGGGTKLELK

SEQ ID NO: 51 - protein, 121 aa, synthetic construct
  REGION 1..121: note = HC variable domain of Hu003_13_F20 antibody
QVQLQESGGGLVKPGGSLKLSCAASGFTFSSYYMSWVRQTPDKRLEWVATISNSGGSTYYPDSVKDRFTISRDNAKNTLYLQMSSLKSEDTAMYYCARDPYYTNYVPMDYWGQGTMVTVSS

SEQ ID NO: 52 - protein, 11 aa, synthetic construct
KASENVGTYVS

SEQ ID NO: 53 - protein, 7 aa, synthetic construct
GASNRYT

SEQ ID NO: 54 - protein, 9 aa, synthetic construct
GQSYSYPLT

SEQ ID NO: 55 - protein, 121 aa, synthetic construct
EVKLVESGGGLVKLGGSLKLSCAASGFTFSSYYMSWVRQTPEKRLEWVATISNSGGSTYYPDSVKDRFTISRDNAKNTLYLQMSSLNSEDTAVYYCARDPYYTNYVPMDYWGQGTSVTVSS

SEQ ID NO: 56 - protein, 107 aa, synthetic construct
NIVMTQSPKSMSMSVGERVTLSCKASENVGTYVSWYQQKPEQSPKLLIYGASNRYTGVPDRFTGSGSATDFTLTISSVQAEDLADYYCGQSYSYPLTFGAGTKLELK

SEQ ID NO: 57 - protein, 121 aa, synthetic construct
EVQLVESGGGLVKPGGSLRLSCAASGFTFSSYYMSWVRQTPEKRLEWVATISNSGGSIYYLDSVKDRFTISRDNAKNSLYLQMNSLRAEDTAVYYCARDPYYSNYVPMDYWGQGTTVTVSS

SEQ ID NO: 58 - protein, 107 aa, synthetic construct
DIVMTQTPSSLSASVGDRVTITCKASQYVDTYVAWYQQKPGKAPKPLIYSASTRHTGVPSRFSGSGSGTDFTLTISSLQPEDFATYFCAQYSSSPLTFGQGTKLELK

SEQ ID NO: 59 - protein, 121 aa, synthetic construct
EVQLVESGGGLVKPGGSLRLSCAASGFTFSSYYMSWVRQTPEKRLEWVATISNSGGSTYYPDSVKDRFTISRDNAKNSLYLQMNSLRAEDTAVYYCARDPYYTNYVPMDYWGQGTTVTVSS

SEQ ID NO: 60 - protein, 107 aa, synthetic construct
DIVMTQSPDSLAVSLGERVTLSCKASENVGTYVSWYQQKPRQPPKLLIYGASNRYTGVPDRFSGSGSGTDFTLTISSLQAEDVALYYCGQSYSYPLTFGQGTRLEIK

SEQ ID NO: 61 - protein, 107 aa, synthetic construct
NIVMTQSPDSLAVSLGERATINCKASENVGTYVSWYQQKPGQPPKLLIYGASNRYTGVPDRFSGSGSGTDFTLTISSLQAEDVAVYYCGQSYSYPLTFGQGTKLEIK

SEQ ID NO: 62 - protein, 120 aa, synthetic construct
QVQLVQSGAEVKKPGASVKVSCKASGYTFTDYYMDWVRQAPGQGLEWLGYIYPNNGGTSYNQKFKGRVTMTTDKSTSTAYMELRSLRSDDTAVYYCARSGYGNYYTMDYWGQGTTVTVSS

SEQ ID NO: 63 - protein, 107 aa, synthetic construct
DIVMTQSPDSLAVSLGERVTINCKASQSVGNNVAWYQQKPGQSPKLLIYYASNRYTGVPDRFSGSGSGTDFTLTISSLQAEDVAVYYCQQHYSSPSTFGQGTKLEIK

SEQ ID NO: 64 - protein, 107 aa, synthetic construct
DIVMTQSQKFMSTSVGDRVSITCKASQSVGNNVAWYQQKPGQSPKLLIYYASNRYTGVPDRFTGSGSGTDFTLTISNMQSEDLADYFCQQHYSSPSTFGGGTKLEIK

SEQ ID NO: 65 - protein, 107 aa, synthetic construct
DIVMTQSPDSLPVSLGERATINCKASQSVGNNVAWYQQKPGQPPKLLIYYASNRYTGVPDRFSGSGSGTDFTLTISSLQAEDVAVYYCQQHYSSPSTFGQGTKLEIK

SEQ ID NO: 66 - protein, 120 aa, synthetic construct
QVQLVQSGAEVKKPGASVKVSCKASGYTFTDYYMDWVRQAPGQGLEWLGYIYPNNGGTSYNQKFKGRVTMTTDKSTSTAYMELRSLRSDDTAVYYCARGGYYSYYSYDYWGQGTTVTVSS

SEQ ID NO: 67 - protein, 107 aa, synthetic construct
DIVMTQSPDSLAVSLGERVTINCKASQSVGNNVAWYQQKPGQSPKLLIYYASNRYTGVPDRFSGSGSGTDFTLTISSLQAEDVAVYYCQQHYSSPYTFGQGTKLEIK

SEQ ID NO: 68 - protein, 107 aa, synthetic construct
DIVMTQSQKFMSTSVGDRVSITCKASQSVGNNVAWYQQKPGQSPKLLIYYASNRYTGVPDRFTGSGSGTDFTLTISNMQSEDLADYFCQQHYSSPYTFGGGTKLEIK

SEQ ID NO: 69 - protein, 107 aa, synthetic construct
DIVMTQSPDSLPVSLGERATINCKASQSVGNNVAWYQQKPGQPPKLLIYYASNRYTGVPDRFSGSGSGTDFTLTISSLQAEDVAVYYCQQHYSSPYTFGQGTKLEIK

SEQ ID NO: 70 - protein, 120 aa, synthetic construct
QVQLVQSGAEVKKPGASVKVSCKASGYTFTDYYMDWVRQAPGQGLEWLGYIYPNNGGTSYNQKFKGRVTMTTDKSTSTAYMELRSLRSDDTAVYYCARSGYKAYYAMDYWGQGTTVTVSS

SEQ ID NO: 71 - protein, 107 aa, synthetic construct; identical to SEQ ID NO: 67

SEQ ID NO: 72 - protein, 107 aa, synthetic construct; identical to SEQ ID NO: 68

SEQ ID NO: 73 - protein, 107 aa, synthetic construct; identical to SEQ ID NO: 69

SEQ ID NO: 74 - protein, 17 aa, synthetic construct
YIYPNNAGTSYNQKFKG

SEQ ID NO: 75 - protein, 120 aa, synthetic construct
QVQLVQSGAEVKKPGASVKVSCKASGYTFTDYYMDWVRQAPGQGLEWLGYIYPNNAGTSYNQKFKGRVTMTTDKSTSTAYMELRSLRSDDTAVYYCARSGYGNYYTMDYWGQGTTVTVSS

SEQ ID NO: 76 - protein, 17 aa, synthetic construct
YIYPNKGGTSYNQKFKG

SEQ ID NO: 77 - protein, 120 aa, synthetic construct
QVQLVQSGAEVKKPGASVKVSCKASGYTFTDYYMDWVRQAPGQGLEWLGYIYPNKGGTSYNQKFKGRVTMTTDKSTSTAYMELRSLRSDDTAVYYCARSGYGNYYTMDYWGQGTTVTVSS

SEQ ID NO: 78 - protein, 17 aa, synthetic construct
YIYPNNAGTSYNQKFKG

SEQ ID NO: 79 - protein, 120 aa, synthetic construct
QVQLVQSGAEVKKPGASVKVSCKASGYTFTDYYMDWVRQAPGQGLEWLGYIYPNNAGTSYNQKFKGRVTMTTDKSTSTAYMELRSLRSDDTAVYYCARGGYYSYYSYDYWGQGTTVTVSS

SEQ ID NO: 80 - protein, 17 aa, synthetic construct
YIYPNKGGTSYNQKFKG

SEQ ID NO: 81 - protein, 120 aa, synthetic construct
QVQLVQSGAEVKKPGASVKVSCKASGYTFTDYYMDWVRQAPGQGLEWLGYIYPNKGGTSYNQKFKGRVTMTTDKSTSTAYMELRSLRSDDTAVYYCARGGYYSYYSYDYWGQGTTVTVSS

SEQ ID NO: 82 - protein, 17 aa, synthetic construct
YIYPNNAGTSYNQKFKG

SEQ ID NO: 83 - protein, 120 aa, synthetic construct
QVQLVQSGAEVKKPGASVKVSCKASGYTFTDYYMDWVRQAPGQGLEWLGYIYPNNAGTSYNQKFKGRVTMTTDKSTSTAYMELRSLRSDDTAVYYCARSGYKAYYAMDYWGQGTTVTVSS

SEQ ID NO: 84 - protein, 17 aa, synthetic construct
YIYPNKGGTSYNQKFKG

SEQ ID NO: 85 - protein, 120 aa, synthetic construct
QVQLVQSGAEVKKPGASVKVSCKASGYTFTDYYMDWVRQAPGQGLEWLGYIYPNKGGTSYNQKFKGRVTMTTDKSTSTAYMELRSLRSDDTAVYYCARSGYKAYYAMDYWGQGTTVTVSS

SEQ ID NO: 86 - protein, 460 aa, synthetic construct
METDTLLLWVLLLWVPGSTGDSEVEYRAEVGQNAYLPCFYTPAAPGNLVPVCWGKGACPVFECGNVVLRTDERDVNYWTSRYWLNGDFRKGDVSLTIENVTLADSGIYCCRIQIPGIMNDEKFNLKLVIKPAKVTPAPTLQRDFTAAFPRMLTTRGHGPAETQTLGSLPDINLTQISTLANELRDSRLANDLRDSGATIRIEGRMDPKSCDKTHTCPPCPAPELLGGPSVFLFPPKPKDTLMISRTPEVTCVVVDVSHEDPEVKFNWYVDGVEVHNAKTKPREEQYNSTYRVVSVLTVLHQDWLNGKEYKCKVSNKALPAPIEKTISKAKGQPREPQVYTLPPSREEMTKNQVSLTCLVKGFYPSDIAVEWESNGQPENNYKTTPPVLDSDGSFFLYSKLTVDKSRWQQGNVFSCSVMHEALHNHYTQKSLSLSPGKGGGLNDIFEAQKIEWHEHHHHHH

SEQ ID NO: 87 - protein, 128 aa, synthetic construct
MAHHHHHHSAALEVLFQGPSEVEYRAEVGQNAYLPCFYTPAAPGNLVPVCWGKGACPVFECGNVVLRTDERDVNYWTSRYWLNGDFRKGDVSLTIENVTLADSGIYCCRIQIPGIMNDEKFNLKLVIK

SEQ ID NO: 88 - protein, 119 aa, synthetic construct
MSEVEYRAEVGQNAYLPCFYTPAAPGNLVPVCWGKGACPVFECGNVVLRTDERDVNYWTSRYWLNGDFRKGDVSLTIENVTLADSGIYCCRIQIPGIMNDEKFNLKLVIKGGGGSEPEA